European Patent Specification EP 3 346 014 B1, published November 8, 2023. Title: A Method For Detecting Oral Precancerous Conditions. Applicant: Kagoshima University. The sequence listing filed with the application follows.

SEQUENCE LISTING (30 sequences)

SEQ ID NO: 1 - DNA, 36 bp, Artificial
  probe
cagaggggaagaggaaagaggaagaagcgctcagat

SEQ ID NO: 2 - DNA, 43 bp, Artificial
  probe
gctccgcggctgtcgtgaaggttaaaaccgaaaataaaaatgg

SEQ ID NO: 3 - DNA, 24 bp, Artificial
  probe
cgcgaggatctggagcgaactgct

SEQ ID NO: 4 - DNA, 31 bp, Artificial
  probe
gcgcctcggtgggccgctcccttccctccct

SEQ ID NO: 5 - DNA, 21 bp, Artificial
  probe
ctcctttcgcccgcgccctcc

SEQ ID NO: 6 - DNA, 34 bp, Artificial
  probe
gttcgctccggacaccatggacaagttttggtgg

SEQ ID NO: 7 - DNA, 23 bp, Artificial
  probe
cagtccctgcacccaggtttcca

SEQ ID NO: 8 - DNA, 32 bp, Artificial
  probe
ttgcgcggctctcctcagctccttcccgccgc

SEQ ID NO: 9 - DNA, 27 bp, Artificial
  probe
ggagggaggaggcgagaggagtcggga

SEQ ID NO: 10 - DNA, 37 bp, Artificial
  probe
tctgcgctgcagccaccgccgcggttgatactacttt

SEQ ID NO: 11 - DNA, 26 bp, Artificial
  probe
cctggagcccgagtccttgcacgcca

SEQ ID NO: 12 - DNA, 41 bp, Artificial
  probe
ggcgcccgggagaacactttttccttgatccggggaaagca

SEQ ID NO: 13 - DNA, 22 bp, Artificial
  probe
cgcgagagtaggcgcgtggagg

SEQ ID NO: 14 - DNA, 38 bp, Artificial
  probe
gcgctcggccatctttgatcctgaccaggcgacttcgt

SEQ ID NO: 15 - DNA, 21 bp, Artificial
  probe
cgcgggtctgggtttccacgc

SEQ ID NO: 16 - DNA, 31 bp, Artificial
  probe
gcgtcaggtcatcaccccggagcccagtggg

SEQ ID NO: 17 - DNA, 21 bp, Artificial
  probe
cagcccctgcgcgctcctaga

SEQ ID NO: 18 - DNA, 34 bp, Artificial
  probe
gctcgggccgtggctcgtcggggtctgtgtcttt

SEQ ID NO: 19 - DNA, 29 bp, Artificial
  probe
cgggagaagcgtgaggggacagatttgtg

SEQ ID NO: 20 - DNA, 40 bp, Artificial
  probe
accggcgcggtttttgtcagcttactccggccaaaaaaga

SEQ ID NO: 21 - DNA, 24 bp, Artificial
  probe
ccgctccagataagagtgtgcgga

SEQ ID NO: 22 - DNA, 31 bp, Artificial
  probe
aagcgcggcggggctgagacgcgaccaggac

SEQ ID NO: 23 - DNA, 24 bp, Artificial
  probe
gttctcagataactgggcccctgc

SEQ ID NO: 24 - DNA, 37 bp, Artificial
  probe
gctcaggaggccttcaccctctgctctgggtaaaggt

SEQ ID NO: 25 - DNA, 27 bp, Artificial
  probe
ctttccaataaagcatgtccagcgctc

SEQ ID NO: 26 - DNA, 37 bp, Artificial
  probe
gggctttagtttgcacgtccatgaattgtctgccaca

SEQ ID NO: 27 - DNA, 21 bp, Artificial
  probe
ccgccggcttgtgcgctcgct

SEQ ID NO: 28 - DNA, 37 bp, Artificial
  probe
gcctgcctctctggctgtctgcttttgcagggctgct

SEQ ID NO: 29 - DNA, 23 bp, Artificial
  probe
ctgcgacagctcctggaagccgg

SEQ ID NO: 30 - DNA, 34 bp, Artificial
  probe
cgcggatcccaacggagtcaaccgtttcgggagg